European Patent Application EP 4 245 854 A1, published September 20, 2023. Title: miR-29a-like nucleic acid regent, hepatic fibrosis inhibitor and pharmaceutical composition. Applicant: Tokyo medical university. The sequence listing filed with the application follows.

SEQUENCE LISTING (4 sequences)

SEQ ID NO: 1 - DNA, 16 bp, Artificial Sequence
  miR-29a-like nucleic acid
uagcaccaggctgucc

SEQ ID NO: 2 - DNA, 16 bp, Artificial Sequence
  miR-29a-like nucleic acid
uagcaccaggctgucc

SEQ ID NO: 3 - DNA, 16 bp, Artificial Sequence
  mi-29a-like ncleic acid
tagcaccaggctgtcc

SEQ ID NO: 4 - DNA, 16 bp, Artificial Sequence
  miR-29a-like nucleic acid
tagcaccaggctgtcc